European Patent Specification EP 4 114 966 B1, published February 26, 2025. Title: METHODS AND COMPOSITIONS FOR SEQUENCING DOUBLE STRANDED NUCLEIC ACIDS. Applicant: OMNIOME, Inc. Subramanian, Hari K.K. Feldman, Aaron W. Chen, Chih-Yuan Malyshev, Denis Richmond, Greg. The sequence listing filed with the application follows.

SEQUENCE LISTING (9 sequences)

SEQ ID NO: 1 - protein, 10 aa, Artificial Sequence
  Synthetic Polypeptide
EQKLISEEDL

SEQ ID NO: 2 - protein, 26 aa, Artificial Sequence
  Synthetic Polypeptide
KRRWKKNFIAVSAANRFKKISSSGAL

SEQ ID NO: 3 - protein, 7 aa, Artificial Sequence
  Synthetic Polypeptide
DYKDDDD

SEQ ID NO: 4 - protein, 8 aa, Artificial Sequence
  Synthetic Polypeptide
DYKDDDDK

SEQ ID NO: 5 - protein, 7 aa, Artificial Sequence
  Synthetic Polypeptide
DYKDDDK

SEQ ID NO: 6 - DNA, 26 bp, Artificial Sequence
  Synthetic Oligonucleotide
  misc_feature (24)..(25): phosphorothiate bond
  misc_feature (25)..(26): phosphorothiate bond
cgccgtatcattcaagcagaagacgg

SEQ ID NO: 7 - DNA, 24 bp, Artificial Sequence
  Synthetic Oligonucleotide
  misc_feature (23)..(24): phosphorothiate bond
atctcgtatgccgtcttctgcttg

SEQ ID NO: 8 - DNA, 28 bp, Artificial Sequence
  Synthetic Oligonucleotide
gtgactggagttcagacgtgtgctcttc

SEQ ID NO: 9 - DNA, 67 bp, Artificial Sequence
  Synthetic Oligonucleotide
cggcgaccaccgagatcggcgaccaccgagatctacactctttccctacacgacgctcttccgatct